European Patent Specification EP 3 807 294 B1, published January 14, 2026. Title: Peptides Having Antiperspirant Activity. Applicant: AZIENDE CHIMICHE RIUNITE ANGELINI FRANCESCO - A.C.R.A.F. S.P.A. The sequence listing filed with the application follows.

SEQUENCE LISTING (10 sequences)

SEQ ID NO: 1 - protein, 4 aa, Artificial Sequence
  None
WMRL

SEQ ID NO: 2 - protein, 5 aa, Artificial Sequence
  None
WMRLK

SEQ ID NO: 3 - protein, 6 aa, Artificial Sequence
  None
WMRLKA

SEQ ID NO: 4 - protein, 6 aa, Artificial Sequence
  None
WMNLKT

SEQ ID NO: 5 - protein, 5 aa, Artificial Sequence
  None
WMFLK

SEQ ID NO: 6 - protein, 12 aa, Artificial Sequence
  None
RMYKMMAGMYLR

SEQ ID NO: 7 - protein, 11 aa, Artificial Sequence
  None
RVMYKMNKRDY

SEQ ID NO: 8 - protein, 11 aa, Artificial Sequence
  None
RVMFKMFKRDY

SEQ ID NO: 9 - protein, 15 aa, Artificial Sequence
  None
RMTMLMLDFKYMKWW

SEQ ID NO: 10 - protein, 15 aa, Artificial Sequence
  None
KMTMRMLYFKYMMWW